European Patent Application EP 4 700 041 A1, published February 25, 2026. Title: Novel Peptide Having Activity of Retarding Degradation of Hyaluronic Acid and Uses Thereof. Applicant: CAREGEN CO., LTD. The sequence listing filed with the application follows.

SEQUENCE LISTING (1 sequence)

SEQ ID NO: 1 - protein, 12 aa, synthetic construct
KIWNLEPSRNGT